European Patent Application EP 4 545 645 A1, published April 30, 2025. Title: Verfahren zur Herstellung einer wässerigen Lösung enthaltend Glycolsäure. Applicant: Annikki GmbH. The sequence listing filed with the application follows.

SEQUENCE LISTING (18 sequences)

SEQ ID NO: 1 - protein, 337 aa, Geobacillus stearothermophilus
MKAAVVEQFKKPLQVKEVEKPKISYGEVLVRIKACGVCHTDLHAAHGDWPVKPKLPLIPGHEGVGVIEEVGPGVTHLKVGDRVGIPWLYSACGHCDYCLSGQETLCERQQNAGYSVDGGYAEYCRAAADYVVKIPDNLSFEEAAPIFCAGVTTYKALKVTGAKPGEWVAIYGIGGLGHVAVQYAKAMGLNVVAVDLGDEKLELAKQLGADLVVNPKHDDAAQWIKEKVGGVHATVVTAVSKAAFESAYKSIRRGGACVLVGLPPEEIPIPIFDTVLNGVKIIGSIVGTRKDLQEALQFAAEGKVKTIVEVQPLENINDVFDRMLKGQINGRVVLKVD

SEQ ID NO: 2 - DNA, 1014 bp, Geobacillus stearothermophilus
  source 1..1014: mol_type = genomic DNA
atgaaagctgcagttgtggaacaatttaaaaagccgttacaagtgaaagaagtggaaaaacctaagatctcatacggggaagtattagtgcgcatcaaagcgtgtggggtatgccatacagacttgcatgccgcacatggcgactggcctgtaaagcctaaactgcctctcattcctggccatgaaggcgtcggtgtaattgaagaagtaggtcctggggtaacacatttaaaagttggagatcgcgtaggtatcccttggctttattcggcgtgcggtcattgtgactattgcttaagcggacaagaaacattatgcgaacgtcaacaaaacgctggctattccgtcgatggtggttatgctgaatattgccgtgctgcagccgattatgtcgtaaaaattcctgataacttatcgtttgaagaagccgctccaatcttttgcgctggtgtaacaacatataaagcgctcaaagtaacaggcgcaaaaccaggtgaatgggtagccatttacggtatcggcgggcttggacatgtcgcagtccaatacgcaaaggcgatggggttaaacgtcgttgctgtcgatttaggtgatgaaaaacttgagcttgctaaacaacttggtgcagatcttgtcgtcaatccgaaacatgatgatgcagcacaatggataaaagaaaaagtgggcggtgtgcatgcgactgtcgtcacagctgtttcaaaagccgcgttcgaatcagcctacaaatccattcgtcgcggtggtgcttgcgtactcgtcggattaccgccggaagaaatacctattccaattttcgatacagtattaaatggagtaaaaattattggttctatcgttggtacgcgcaaagacttacaagaggcacttcaatttgcagcagaaggaaaagtaaaaacaattgtcgaagtgcaaccgcttgaaaacattaacgacgtattcgatcgtatgttaaaagggcaaattaacggccgcgtcgtgttaaaagtagattaa

SEQ ID NO: 3 - protein, 342 aa, Acetobacter pasteurianus
MSGKMKAAVVHEFGKPLTIEELDIPTIKPTQILVKMIACGVCHTDLHAASGDWPKKPHLPFIPGHEGVGTVVQVGSEVDWVKEGDVVGVPWLYSACGHCEHCLAGWETLCAKQEETGYSVNGCFAEYVVADPNYIAHLPKGVDPVKVAPVLCAGLTVYKGLKMTDTRAGNWVAISGVGGLGQMAVQYAVAMGLNVVAVDIDDEKLATAKKLGATYTVNARNTDPAAFMQEKVGGVHGGLITAVSTKAFSQAMGYVRAGGTLVLNGLPPGDFPISIFDVVMNAITIRGSIVGTRLDMIEALSFFAEGKVTSVTTTDRIDNINAIFDALKNGRVEGRVVLDFRN

SEQ ID NO: 4 - DNA, 1029 bp, Acetobacter pasteurianus
  source 1..1029: mol_type = genomic DNA
atgtccggaaaaatgaaagccgctgtggttcatgaatttggcaaaccactgaccattgaagaactggacattcccaccattaaacccacccagattttggttaaaatgattgcctgcggcgtgtgccatacagatttgcatgctgccagcggggattggcccaaaaaaccacatctgccgtttattcccggccacgaaggcgttggcacggttgtgcaggttggcagcgaagtagactgggtaaaggaaggcgacgttgttggcgtgccttggctctattctgcctgcggccattgcgagcattgtctggctgggtgggaaaccctttgtgcgaagcaagaagaaaccggctattccgtaaacggctgctttgccgaatacgtggtagcagaccctaactacattgctcatcttcccaaaggcgtagaccctgtaaaagttgcccccgtactgtgcgcaggcctgaccgtttataagggcctgaaaatgacagacacgcgggcagggaactgggttgccatttccggcgttggggggttaggccagatggctgtgcagtacgccgtagcaatggggctgaatgttgtggcggtagatattgatgatgaaaaactggcaaccgccaaaaagcttggtgcaacgtacactgttaacgccagaaatacagatccggcagcatttatgcaggaaaaagttggtggcgtacacggtggattgatcaccgctgtttccaccaaagcattttctcaggctatgggttatgtgcgggcagggggcactttggtgctaaatgggctgccgccgggtgatttcccaatttctatctttgacgtggtcatgaatgccattaccattcgcggctccatagtaggcacacggctggacatgattgaagctctttccttctttgcggaagggaaggtaacatctgtcaccacaacggatcggattgataacatcaacgcaatttttgatgcgctcaagaacggtcgggtggaaggccgcgtggttctggacttccgcaactga

SEQ ID NO: 5 - protein, 342 aa, Achromobacter xylosoxidans
MNKTMKAAVARAFGKPLEIEEVEVPRPRAGELLVKIEACGVCHTDLHAVEGDWPVKPNPPFIPGHEGVGHVVAVGEGVTHVKEGDRVGIPWLYSACGHCEHCLGGWETLCEQQQNAGYSVNGGFAEYALAAADYVGLLPKNVGFVDIAPVLCAGVTVYKGLKMTDTRPGNWVVVSGIGGLGHMAVQYARAMGLNVAAVDIDDDKLDFAKRLGAEVVVNAKATDPAAYLKKEIGGAHGALITAVSPKAFEQALGMVRRGGTVALNGLPPGDFPLSIFDMVLNGVTVRGSIVGSRLDLQESLQFAEEGKVRATVATEKLENINSVFDRMRRGQIEGRIVLDMAA

SEQ ID NO: 6 - DNA, 1029 bp, Achromobacter xylosoxidans
  source 1..1029: mol_type = genomic DNA
atgaacaagaccatgaaggccgcggtggcccgcgcgttcggcaaacccctggaaatcgaagaagtcgaggtgccgcgcccgcgcgcgggcgaactgttggtgaagatcgaggcctgcggcgtctgccacaccgatctgcacgcggtcgagggcgactggccggtcaagcccaatccccctttcatcccgggccacgaaggcgtgggccacgtggtggcggtgggcgaaggcgtgacgcacgtcaaggaaggcgaccgcgtcggcatcccctggctgtattccgcctgtggccattgcgagcattgcctgggcggctgggagacgctgtgcgaacagcagcagaacgccggctactccgtcaacggcggcttcgccgagtacgcgctggccgcggccgactacgtgggcctgctgccgaagaatgtcggcttcgtcgacatcgccccggtactgtgcgccggcgtcacggtctacaaaggcctgaagatgacggacacacggccaggcaactgggtcgtggtctccggcatcggcggcctgggccacatggcggtgcagtatgcgcgcgccatgggcttgaacgtggcggccgtggacatcgacgacgacaaactggatttcgccaagcgtctcggcgccgaggtggtcgtgaatgccaaggccaccgatccagcggcttacctgaagaaggaaatcggcggcgcccacggcgcgctgatcacggcggtttcgcccaaggccttcgagcaggcgctgggcatggtgcgtcgcggcggcacggtggcgctcaacggcctgccgccgggcgacttcccgctgtcgatcttcgacatggtgctcaacggcgtgacggtgcgcggttcgatcgtgggttcgcgcctggacttgcaggaatcgctgcagttcgccgaggaaggcaaggtgcgcgcgaccgtggcgaccgagaagctggagaacatcaacagcgtgttcgaccgcatgcgccgcggccagatcgaaggccgcatcgtgctggacatggcggcgtaa

SEQ ID NO: 7 - protein, 451 aa, Carnobacterium divergens
MKVVVVGCTHAGTAAVKTILNEHPDASVSVYERNDNVSFLSCGIALYVGGVVKDPAGLFYSSPEELASMGAKINMEHNVKNIDNENKVVVIENLKTGETFEESYDKLVMTTGSWPIIPPIDGINSENILLCKNYNQANEIIKESKNAKKIVIVGGGYIGIELVEAFAESGKQVTLVDGLDRILNKYLDAEFTSVLEHDLQERGVTLALNQTVEKFVANESGAVTAVKTPVGEYEADLVILCVGFKPNTDLLKDKVEMLPNGAIVVDEYMRTSDEAIFAAGDSCAVHYNPTGGSAYIPLATNAVRMGALVGKNIVSPTVKYRGTQATSGLYLFGFNIGSTGLTENSAPHFGVEVRSVVVEDNYRPEFMPTTEKVTMKLVYEVGTNRIVGGQIMSKYDVTQSANTLSLCVQNKMTIEDLAYVDFFFQPHFDRPWNYLNILAQAAVEQERKLAK

SEQ ID NO: 8 - DNA, 1356 bp, Carnobacterium divergens
  source 1..1356: mol_type = genomic DNA
atgaaagtagtagtagtaggctgtacacatgcaggaacagcggcagttaagacgattttaaatgaacatccagatgcatcagtatcagtatatgagcgtaatgacaatgtctcatttctatcttgtgggattgcgttgtatgttggtggagttgtgaaagatcctgcaggtttgttttattcaagtccagaagaacttgcatcaatgggcgcgaaaattaacatggaacacaatgtgaaaaatatagataatgagaataaggtcgtagtaattgagaatttaaaaacaggcgaaacatttgaagaaagctatgataagttggtaatgacaactggatcatggccaattattcctccaattgatggaatcaatagtgaaaatattcttttgtgtaaaaactataaccaagcaaatgaaattattaaagaatcaaaaaatgctaaaaagattgtcattgttggtggtggctatattggaattgaattagttgaggcatttgcagaatctggcaagcaagtgacgctagttgatggattagatcgtattttaaacaaatatttagatgctgaattcacttctgttttagagcatgatttacaagaaagaggcgttacgctagctttaaaccaaaccgtcgagaaatttgttgccaatgaatcaggtgctgtgacagctgtgaaaacaccagttggagaatatgaggctgatttagttattttatgtgttggatttaaaccaaatactgatttgttgaaggataaagtagagatgttgccaaatggtgccatcgtagtggatgaatatatgagaacaagcgatgaagcgatttttgctgctggcgatagttgcgcggttcattataatccaactggaggctctgcgtatattccgttagctacaaatgcagttagaatgggagctttagttgggaaaaatattgtttctccaacagttaaatatcgtggcacgcaagcaacttctggtttatatttatttggttttaatataggttcaaccggattgactgaaaatagcgctcctcattttggcgtagaggttcgttcagtagttgtagaagataattatcgtccagagtttatgccgacaacagagaaagtaacgatgaaattagtttatgaagtaggaacgaatcggattgttggaggtcaaatcatgtcaaaatatgatgtgacacaatctgccaatacgttatctttatgtgttcaaaataaaatgacgattgaggatttggcttatgtagatttcttcttccaacctcactttgatcgtccttggaactatttaaatattttagcgcaagcagctgttgagcaagagcgtaaactagcaaaataa

SEQ ID NO: 9 - protein, 457 aa, Streptococcus mutans
MSKIVIVGANHAGTAAINTILDNYGSENEVVVFDQNSNISFLGCGMALWIGKQISGPQGLFYADKESLEAKGAKIYMESPVTAIDYDAKRVTALVNGQEHVESYEKLILATGSTPILPPIKGAAIKEGSRDFEATLKNLQFVKLYQNAEDVINKLQDKSQNLNRIAVVGAGYIGVELAEAFKRLGKEVILIDVVDTCLAGYYDQDLSEMMRQNLEDHGIELAFGETVKAIEGDGKVERIVTDKASHDVDMVILAVGFRPNTALGNAKLKTFRNGAFLVDKKQETSIPDVYAIGDCATVYDNAINDTNYIALASNALRSGIVAGHNAAGHKLESLGVQGSNGISIFGLNMVSTGLTQEKAKRFGYNPEVTAFTDFQKASFIEHDNYPVTLKIVYDKDSRLVLGAQMASKEDMSMGIHMFSLAIQEKVTIERLALLDYFFLPHFNQPYNYMTKAALKAK

SEQ ID NO: 10 - DNA, 1374 bp, Streptococcus mutans
  source 1..1374: mol_type = genomic DNA
atgagcaaaattgttatcgtgggtgcaaatcatgcaggcaccgcagcaattaataccattctggataattatggcagcgaaaatgaagtggttgtgtttgatcagaatagcaacattagctttctgggttgtggtatggcactgtggattggtaaacaaattagcggtccgcagggtctgttttatgcagataaagaaagcctggaagcaaaaggtgccaaaatctatatggaaagtccggttaccgccattgattatgatgcaaaacgtgttaccgcactggttaatggtcaagaacatgttgaaagctacgagaaactgattctggcaaccggtagcaccccgattctgcctccgattaaaggtgcagccattaaagaaggtagtcgcgattttgaagcaaccctgaaaaatctgcagttcgtgaaactgtatcagaatgccgaagatgtgattaacaaactgcaggataaaagccagaatctgaatcgtattgcagttgttggtgcaggttatattggtgttgaactggcagaagcatttaaacgtctgggtaaagaagtgattctgattgacgttgttgatacctgtctggcaggttattatgatcaggatctgagcgaaatgatgcgtcagaatctggaagatcatggtatcgaactggcatttggtgaaaccgttaaagcaattgaaggtgatggtaaagtggaacgtattgttaccgataaagcaagccatgatgtggatatggttattctggcagttggttttcgtccgaatacagcactgggtaatgcaaaactgaaaacctttcgtaatggtgcctttctggtggataaaaaacaagaaaccagcatcccggatgtttatgcaattggtgattgtgcaaccgtgtatgataatgccattaacgacaccaactatattgcactggcaagcaatgcactgcgtagcggtattgttgcaggtcataatgcagccggtcataaactggaaagtctgggtgttcagggtagcaatggtatttcaatttttggcctgaatatggttagcaccggtctgacccaagaaaaagccaaacgttttggttataatccggaagttaccgcctttaccgattttcagaaagccagctttatcgagcatgataactatccggttacgctgaaaattgtgtatgacaaagatagccgtctggttctgggtgcacagatggccagcaaagaagatatgagcatgggtattcacatgtttagcctggccattcaagagaaagttaccattgaacgtctggccctgctggattatttctttctgccgcattttaatcagccgtacaactatatgaccaaagcagcactgaaagccaaataa

SEQ ID NO: 11 - protein, 451 aa, synthetic construct
  source 1..451: note = variant of SEQ ID No. 7
MKVVVVGCTHAGTAAVKTILNEHPDASVSVYERNDNVSFLSCGIALYVGGVVKDPAGLFYSSPEELASMGAKINMEHNVKNIDNENKVVVIENLKTGETFEESYDKLVMTTGSWPIIPPIDGINSENILLCKNYNQANEIIKESKNAKKIVIVGGGYIGIELVEAFAESGKQVTLVARSDRILRKYLDAEFTSVLEHDLQERGVTLALNQTVEKFVANESGAVTAVKTPVGEYEADLVILCVGFKPNTDLLKDKVEMLPNGAIVVDEYMRTSDEAIFAAGDSCAVHYNPTGGSAYIPLATNAVRMGALVGKNIVSPTVKYRGTQATSGLYLFGFNIGSTGLTENSAPHFGVEVRSVVVEDNYRPEFMPTTEKVTMKLVYEVGTNRIVGGQIMSKYDVTQSANTLSLCVQNKMTIEDLAYVDFFFQPHFDRPWNYLNILAQAAVEQERKLAK

SEQ ID NO: 12 - DNA, 1356 bp, synthetic construct
  source 1..1356: mol_type = other DNA; note = variant of SEQ ID No. 8
atgaaagtagtagtagtaggctgtacacatgcaggaacagcggcagttaagacgattttaaatgaacatccagatgcatcagtatcagtatatgagcgtaatgacaatgtctcatttctatcttgtgggattgcgttgtatgttggtggagttgtgaaagatcctgcaggtttgttttattcaagtccagaagaacttgcatcaatgggcgcgaaaattaacatggaacacaatgtgaaaaatatagataatgagaataaggtcgtagtaattgagaatttaaaaacaggcgaaacatttgaagaaagctatgataagttggtaatgacaactggatcatggccaattattcctccaattgatggaatcaatagtgaaaatattcttttgtgtaaaaactataaccaagcaaatgaaattattaaagaatcaaaaaatgctaaaaagattgtcattgttggtggtggctatattggaattgaattagttgaggcatttgcagaatctggcaagcaagtgacgctagttgcgcgtagcgatcgtattttacgtaaatatttagatgctgaattcacttctgttttagagcatgatttacaagaaagaggcgttacgctagctttaaaccaaaccgtcgagaaatttgttgccaatgaatcaggtgctgtgacagctgtgaaaacaccagttggagaatatgaggctgatttagttattttatgtgttggatttaaaccaaatactgatttgttgaaggataaagtagagatgttgccaaatggtgccatcgtagtggatgaatatatgagaacaagcgatgaagcgatttttgctgctggcgatagttgcgcggttcattataatccaactggaggctctgcgtatattccgttagctacaaatgcagttagaatgggagctttagttgggaaaaatattgtttctccaacagttaaatatcgtggcacgcaagcaacttctggtttatatttatttggttttaatataggttcaaccggattgactgaaaatagcgctcctcattttggcgtagaggttcgttcagtagttgtagaagataattatcgtccagagtttatgccgacaacagagaaagtaacgatgaaattagtttatgaagtaggaacgaatcggattgttggaggtcaaatcatgtcaaaatatgatgtgacacaatctgccaatacgttatctttatgtgttcaaaataaaatgacgattgaggatttggcttatgtagatttcttcttccaacctcactttgatcgtccttggaactatttaaatattttagcgcaagcagctgttgagcaagagcgtaaactagcaaaataa

SEQ ID NO: 13 - protein, 451 aa, synthetic construct
  source 1..451: note = variant of SEQ ID No. 7
MKVVVVGCTHAGTAAVKTILNEHPDASVSVYERNDNVSFLSCGIALYVGGVVKDPAGLFYSSPEELASMGAKINMEHNVKNIDNENKVVVIENLKTGETFEESYDKLVMTTGSWPIIPPIDGINSENILLCKNYNQANEIIKESKNAKKIVIVGGGYIAIELVEAFAESGKQVTLVARSDRILRKYLDAEFTSVLEHDLQERGVTLALNQTVEKFVANESGAVTAVKTPVGEYEADLVILCVGFKPNTDLLKDKVEMLPNGAIVVDEYMRTSDEAIFAAGDSCAVHYNPTGGSAYIPLATNAVRMGALVGKNIVSPTVKYRGTQATSGLYLFGFNIGSTGLTENSAPHFGVEVRSVVVEDNYRPEFMPTTEKVTMKLVYEVGTNRIVGGQIMSKYDVTQSANTLSLCVQNKMTIEDLAYVDFFFQPHFDRPWNYLNILAQAAVEQERKLAK

SEQ ID NO: 14 - DNA, 1356 bp, synthetic construct
  source 1..1356: mol_type = other DNA; note = variant of SEQ ID No. 8
atgaaagtagtagtagtaggctgtacacatgcaggaacagcggcagttaagacgattttaaatgaacatccagatgcatcagtatcagtatatgagcgtaatgacaatgtctcatttctatcttgtgggattgcgttgtatgttggtggagttgtgaaagatcctgcaggtttgttttattcaagtccagaagaacttgcatcaatgggcgcgaaaattaacatggaacacaatgtgaaaaatatagataatgagaataaggtcgtagtaattgagaatttaaaaacaggcgaaacatttgaagaaagctatgataagttggtaatgacaactggatcatggccaattattcctccaattgatggaatcaatagtgaaaatattcttttgtgtaaaaactataaccaagcaaatgaaattattaaagaatcaaaaaatgctaaaaagattgtcattgttggtggtggctatattgcgattgaattagttgaggcatttgcagaatctggcaagcaagtgacgctagttgcgcgtagcgatcgtattttacgtaaatatttagatgctgaattcacttctgttttagagcatgatttacaagaaagaggcgttacgctagctttaaaccaaaccgtcgagaaatttgttgccaatgaatcaggtgctgtgacagctgtgaaaacaccagttggagaatatgaggctgatttagttattttatgtgttggatttaaaccaaatactgatttgttgaaggataaagtagagatgttgccaaatggtgccatcgtagtggatgaatatatgagaacaagcgatgaagcgatttttgctgctggcgatagttgcgcggttcattataatccaactggaggctctgcgtatattccgttagctacaaatgcagttagaatgggagctttagttgggaaaaatattgtttctccaacagttaaatatcgtggcacgcaagcaacttctggtttatatttatttggttttaatataggttcaaccggattgactgaaaatagcgctcctcattttggcgtagaggttcgttcagtagttgtagaagataattatcgtccagagtttatgccgacaacagagaaagtaacgatgaaattagtttatgaagtaggaacgaatcggattgttggaggtcaaatcatgtcaaaatatgatgtgacacaatctgccaatacgttatctttatgtgttcaaaataaaatgacgattgaggatttggcttatgtagatttcttcttccaacctcactttgatcgtccttggaactatttaaatattttagcgcaagcagctgttgagcaagagcgtaaactagcaaaataa

SEQ ID NO: 15 - protein, 451 aa, synthetic construct
  source 1..451: note = variant of SEQ ID No. 7
MKVVVVGCTHAGTAAVKTILNEHPDASVSVYERNDNVSFLSCGIALYVGGVVKDPAGLFYSSPEELASMGAKINMEHNVKNIDNENKVVVIENLKTGETFEESYDKLVMTTGSWPIIPPIDGINSENILLCKNYNQANEIIKESKNAKKIVIVGGGYIGIELVEAFAESNKQVTLVARSDRILRKYLDAEFTSVLEHDLQERGVTLALNQTVEKFVANESGAVTAVKTPVGEYEADLVILCVGFKPNTDLLKDKVEMLPNGAIVVDEYMRTSDEAIFAAGDSCAVHYNPTGGSAYIPLATNAVRMGALVGKNIVSPTVKYRGTQATSGLYLFGFNIGSTGLTENSAPHFGVEVRSVVVEDNYRPEFMPTTEKVTMKLVYEVGTNRIVGGQIMSKYDVTQSANTLSLCVQNKMTIEDLAYVDFFFQPHFDRPWNYLNILAQAAVEQERKLAK

SEQ ID NO: 16 - DNA, 1356 bp, synthetic construct
  source 1..1356: mol_type = other DNA; note = variant of SEQ ID No. 8
atgaaagtagtagtagtaggctgtacacatgcaggaacagcggcagttaagacgattttaaatgaacatccagatgcatcagtatcagtatatgagcgtaatgacaatgtctcatttctatcttgtgggattgcgttgtatgttggtggagttgtgaaagatcctgcaggtttgttttattcaagtccagaagaacttgcatcaatgggcgcgaaaattaacatggaacacaatgtgaaaaatatagataatgagaataaggtcgtagtaattgagaatttaaaaacaggcgaaacatttgaagaaagctatgataagttggtaatgacaactggatcatggccaattattcctccaattgatggaatcaatagtgaaaatattcttttgtgtaaaaactataaccaagcaaatgaaattattaaagaatcaaaaaatgctaaaaagattgtcattgttggtggtggctatattggaattgaattagttgaggcatttgcagaatctaacaagcaagtgacgctagttgcgcgtagcgatcgtattttacgtaaatatttagatgctgaattcacttctgttttagagcatgatttacaagaaagaggcgttacgctagctttaaaccaaaccgtcgagaaatttgttgccaatgaatcaggtgctgtgacagctgtgaaaacaccagttggagaatatgaggctgatttagttattttatgtgttggatttaaaccaaatactgatttgttgaaggataaagtagagatgttgccaaatggtgccatcgtagtggatgaatatatgagaacaagcgatgaagcgatttttgctgctggcgatagttgcgcggttcattataatccaactggaggctctgcgtatattccgttagctacaaatgcagttagaatgggagctttagttgggaaaaatattgtttctccaacagttaaatatcgtggcacgcaagcaacttctggtttatatttatttggttttaatataggttcaaccggattgactgaaaatagcgctcctcattttggcgtagaggttcgttcagtagttgtagaagataattatcgtccagagtttatgccgacaacagagaaagtaacgatgaaattagtttatgaagtaggaacgaatcggattgttggaggtcaaatcatgtcaaaatatgatgtgacacaatctgccaatacgttatctttatgtgttcaaaataaaatgacgattgaggatttggcttatgtagatttcttcttccaacctcactttgatcgtccttggaactatttaaatattttagcgcaagcagctgttgagcaagagcgtaaactagcaaaataa

SEQ ID NO: 17 - protein, 451 aa, synthetic construct
  source 1..451: note = variant of SEQ ID No. 7
MKVVVVGCTHAGTAAVKTILNEHPDASVSVYERNDNVSFLSCGIALYVGGVVKDPAGLFYSSPEELASMGAKINMEHNVKNIDNENKVVVIENLKTGETFEESYDKLVMTTGSWPIIPPIDGINSENILLCKNYNQANEIIKESKNAKKIVIVGGGYIAIELVEAFAESNKQVTLVARSDRILRKYLDAEFTSVLEHDLQERGVTLALNQTVEKFVANESGAVTAVKTPVGEYEADLVILCVGFKPNTDLLKDKVEMLPNGAIVVDEYMRTSDEAIFAAGDSCAVHYNPTGGSAYIPLATNAVRMGALVGKNIVSPTVKYRGTQATSGLYLFGFNIGSTGLTENSAPHFGVEVRSVVVEDNYRPEFMPTTEKVTMKLVYEVGTNRIVGGQIMSKYDVTQSANTLSLCVQNKMTIEDLAYVDFFFQPHFDRPWNYLNILAQAAVEQERKLAK

SEQ ID NO: 18 - DNA, 1356 bp, synthetic construct
  source 1..1356: mol_type = other DNA; note = variant of SEQ ID No. 8
atgaaagtagtagtagtaggctgtacacatgcaggaacagcggcagttaagacgattttaaatgaacatccagatgcatcagtatcagtatatgagcgtaatgacaatgtctcatttctatcttgtgggattgcgttgtatgttggtggagttgtgaaagatcctgcaggtttgttttattcaagtccagaagaacttgcatcaatgggcgcgaaaattaacatggaacacaatgtgaaaaatatagataatgagaataaggtcgtagtaattgagaatttaaaaacaggcgaaacatttgaagaaagctatgataagttggtaatgacaactggatcatggccaattattcctccaattgatggaatcaatagtgaaaatattcttttgtgtaaaaactataaccaagcaaatgaaattattaaagaatcaaaaaatgctaaaaagattgtcattgttggtggtggctatattgcgattgaattagttgaggcatttgcagaatctaacaagcaagtgacgctagttgcgcgtagcgatcgtattttacgtaaatatttagatgctgaattcacttctgttttagagcatgatttacaagaaagaggcgttacgctagctttaaaccaaaccgtcgagaaatttgttgccaatgaatcaggtgctgtgacagctgtgaaaacaccagttggagaatatgaggctgatttagttattttatgtgttggatttaaaccaaatactgatttgttgaaggataaagtagagatgttgccaaatggtgccatcgtagtggatgaatatatgagaacaagcgatgaagcgatttttgctgctggcgatagttgcgcggttcattataatccaactggaggctctgcgtatattccgttagctacaaatgcagttagaatgggagctttagttgggaaaaatattgtttctccaacagttaaatatcgtggcacgcaagcaacttctggtttatatttatttggttttaatataggttcaaccggattgactgaaaatagcgctcctcattttggcgtagaggttcgttcagtagttgtagaagataattatcgtccagagtttatgccgacaacagagaaagtaacgatgaaattagtttatgaagtaggaacgaatcggattgttggaggtcaaatcatgtcaaaatatgatgtgacacaatctgccaatacgttatctttatgtgttcaaaataaaatgacgattgaggatttggcttatgtagatttcttcttccaacctcactttgatcgtccttggaactatttaaatattttagcgcaagcagctgttgagcaagagcgtaaactagcaaaataa